European Patent Application EP 4 585 608 A1, published July 16, 2025. Title: carrier peptide fragment and use thereof. Applicant: TOAGOSEI CO., LTD. The sequence listing filed with the application follows.

SEQUENCE LISTING (1 sequence)

SEQ ID NO: 1 - protein, 14 aa, synthetic construct
RKLAVYWSTYKRSR